European Patent Application EP 4 640 058 A1, published October 29, 2025. Title: ISOLATED BACTERIOPHAGE AGAINST XYLELLA FASTIDIOSA. Applicant: BIOLINE AGROSCIENCES FRANCE. The sequence listing filed with the application follows.

SEQUENCE LISTING (35 sequences)

SEQ ID NO: 1 - DNA, 42368 bp, unidentified
  source 1..42368: mol_type = genomic DNA
tgcagcgccgacaccagcgtgtcgccgtaaatctcccggtcggtgggcatcttgccgctacgcagcgcgtccaggaacgggtccacgtcgatgtccacgccgcgcgggcgggcgcgggtgtcggtggtggcgccggggatgcgcagcttgaactgctggtacagcgtccaggcgtcggtgccgacgcgctcggccaggttgcgatagaccgactgcaccacgctggcgttctgcctggccagctgttcgtcctggcgcgacagcagctgccccaccacgtcgtcgtacacctggccggccggcccgttctcgcgcgcgtcctgctgctgcgcttcggccagcccttgatcgatggcctgctggatttcttccgacgacaccgccggcagatcgtggcgaccgccgggctgcagcctcacctggtcggccacagccgcgtgcagttccggcgtgaccagggtggcgtacttcgccagcgggatcgccacttcgccgcccgtggcgatggcctcgcgcagggcgtcggaatcgaccaggccgcccaggtccgggccgccctcgctgttggccgactggaacaggcgctgggcgccatcggcagacaggtagatggtgtcctcgccctcgctggtcatgtcgcggatgagcgattcgaagcgggtggcggaacgctcgcgggtcttcgactgcgacgccaggttcaccaggtcgctgatcgcccgctgttcctggtgggcatcgaagcggtcggcgttgtgcatcgccgcgcggcgtgcttccgcgatctgcccgcggccttcggccaggaaggtgggcatttcggccgccgcttccaggaaaatgtccgactggctggtgatcttgccttcgctggccagctgcgcggtggcctcgcccgcggcgccgccgccggcctgcaccgccgcttcgcccgccacgcggccggtgatcgacaccgccgtgcgccggctgttcgcaatgaggcggcccgcgaaaccggcggtcagggcgtcgaacgtgcccacagccacaccgcgcgccagcgccttctgccgtgccttctccatcgccggcttgttgcgcaggaaggccgacaccgctgccgggtcgctggtttccacgccggcatcgcccatcacgtccaggatggtcatgccctgttcggtggcgaaggatccggtgccggccgtgacgcccgccacgacgcggctggccggcatcgccgcggacagcgccagctgcggggcggtgttgcccagcgactgcgccaccacggccatgacggcgcgcgggttcgtgaccacggcgcgcgcaatcttgcccgtgtccttcgtcttctcggcgtcggcgatttcctggaagccggcagcggtcgccgcggtttccacgtcggcggcctgcgcgcggcgcgactggtcggccacgtacacggccgtgcgggcggtgtcgtagtcggccgccgactggtagcccaggccgcgggccacctgttcttcgacggatcgggaattcgcgtcccccaggttcggcagcgggatcaagccgaacccggctttgccctgataccaaccggattggaacttgcccaccatttcgctgaaccacgacgggtccgggctggcgcgcatttccggcccgcgcgcggcggcggccttgcgttccttgtccagatccagggccgactgcggcagcgggagccacggcagcgtttccttcgccgacagcaggccgctgttgaactgccggccaaggcccgccagcacgcccgtgtcgtccttggacagcgccgagtggttagggtcgcccagccaccgcgccaggaccggggacgcgctcgcagcgtcgcccagcgcgtcctgctgctgctgctggtcatactccggcaggttgtccgctacgacgccaggcggcaggccgcgctggtcggccaggcgcatggcccggcccatcgcatcgggatccacctgcggcgccgtgacgccggccgcgcgcgcgcgggcctggtcatcttcggcctgggttgccgcgatgatttccgaatacttccccatgttcagttcgtccccgcgctgttggactgcatccgataccgtgccccaatcctaacgatttcggcttcggtcggttcgcgcccggtggacgcacggaagtcgctgatgatttcggcgcggtcggccgccggcagcgcagcaccgaacccttcgatggcgccagcacgggacagcttgccggggatgtcggtggccacgttgcgcacgacggcgcgcaggatcgaatcggcttccgccggggtaggatccttgccgtgccgctggatgaaggcgcgttcggcctcgcggtacacctgggcaaactgggcgcgctgcaccttgcgttcgtccagcttcttcttcggcggcttggccacgaattcgccttcggcgttgcggttgtcgccggcttcgtccaggcccaggatccgcagccccgattcgatgcgctgggactgggtggcccagtcggcgcgcttcgaaggatcgttcgcctgcttctgcttgcccagcagggtgcccagggtttcggtggaaatgcggtcggccagggcgtggatgtcccggcgcgcgaaggtctgcggcgacagcaccgcttcgcgttccagggtttcgaccagcacggcgtcgtcctgggtgaaggtgccggccaccttgttcttccgcaggttttccagcgtgggcagatggcccttgcgctcggcccaggcgtacacctgggcgcccaggatttcgcgcagcggcgcgttcgggttggtcgcctggttgatcgcggtgtacgcgccttccgacgcggcccggtcctcttcctgccggcgcagatccgacagctggaaccgctcgcggatcttgcccaccactgcggcgcggcggcgagggtccgggatggcctgcgcgcgcgcgatggcgtcggcctcgctcggcggtgcggtgcggcccacctgctgcacgggagcatcgccacgccagcgcgacgcccggcccatgacctcttccacgtatcgggcggtcttcgggttctcggcgcggcgcccgcgcttcacgaccgcggcggcgccgccctcgccagcgaagtgggcggccacggcgaattccacgccgccggtcttggcgcgctgggcaaactcacgggcggcagcgcgcgccgatgcgcgggcatccttccggtcgaacccctgggcgctggtggcgcggtactggaacaggccggtggcgttgtcgccgtcgtccagcacttccgggttgaccgcgttggggttgaagccggattcctgttcggccagggcgtacaggtattcccgcggcacgccagcggcgtcggcctcttcgtccaggatcttggccacggccggcgccgggccgcgccctcgctggccagggtcgcggtatgcctgcggctgcgcgccggccaggatcgcatccgcgtcgtcctgggccgcggcatcggacacgaccgggtacagcaggcggtccaccttggcccggtcttccggggtcatctgatcggcgtagcgttcgaagtaggcctgcgcttcgaacgggcgcgcggtggccatgccttcgatggtctgcgaccgcacgctggacaccaggccgcgttcctcggccttgatgagttcttcgcccatgccatcggcttcgcgccgcgcgcggttcatggccagcagttcgttcgccacacggtcctgccgggagaagtcgccggacacgccagcggacaccgcatcggcgcccaggttgtccacagccgccttctgctcggcggtgatgtagccggaatgttcccggtccatgtagccgttcaggcgtccggccacgctgtcccggaagttcatggccacgccttcgaactgctggcgctgcttcggggtcaggccggcgctgatgctgcccaccgtcttgtccaggtcgggcagcagcacttcgtcggcgcccagggcgttcttgcccttgtacttcgaaatgccgtccgggttgccggggttgaacgtgctggcctcccagtcggacagctgcttgcgcgcagccatcaccgcggtggtgtcgttgcgctcctgttcccgctgggcgtattccagggccgggcgcgcgaagctgccgatggcgccggccagcgcctgggcaccggagtcatcggcgcgcgcggtgttgcgtacctgcggaccctgctggacttcgacctggggcgcggtgacgcgcggaatgatggtggccattacccgtagaaccccccggcgctgctggcgatgctggaaatgccggaaagcaccgtggcggtgcccttggccctggtgttgaagcggtcgatgccggcctggttctggatgttgcgcacctgggagttgaagccccaggcggtgcgcgcggtgttcagccggatggcctgctggtcaacctcgccgaacagcgccgtttcgcccaggatttcggccggcgtcccgatcccggcatcgatcccgtttgccgcgatggcagcgcgctgctggcccatgatcgcgcgcgtgcgccaggtctgttgctgggattcgcggtcgcccatggcctgggctgcagccgcgtcgtcggccgccaggcgcgcgttgttggccgcaatctcggcattcgcttcgccggtcttcttgttggcgtcataggacacatacgtggccgcggcggtggccgctgctgccgcgcccagtgcccaggcggcgccggtcgaaatggtaatcggctcacacatcacacacccctgcggcgatagaagggcaggaacggcaagccgtccacgccataggcaatcggatcgctgaactggaaacccagccagcgcagccagcggatcgctgcgatgttccgctgatccacgaaattgtagagaaggttcgggaactggtcttgcatgtattcgaccacgggttccgacagccgcagcagatccttctgcgcgccatgctggttcagcacgctgctgccgatcatccaggccgaccccatgccgcccatgatggagaacggcgacgccccgaacatgcaggcggggcggccgttgtatatggcggtgaagggttcggcggtgcgttccatgccccgcagcatcgcatccagcgggtcgctgcggctgcacgcccacagttcggccaggtccgccgcccgcgggttctccgcgatggcgtgcgcatgttccacggttgccggcacgatggtggcgcggatcatcccttgcccccggcgccgccggcctggccgttggacgacacggccctggtggtgatcgacaggatttccatgggcagcgggtcatccgacacgatgcgcacgcgcccggcatccacgccccagcctgccgggatgtcgcagtcgaacacgccggttttcagatagggcggctggccgtagggttcgaagcggcgttccttcaccgggtagagcttgtccgtaacgccgccggccttcaccccgcgcgacgccagcagcaggatgctgaccttgtacgccagcttctgctgatcgcgcatcgaatcgccgcccggcgaattcagttccagggtttcgacctcgcaggcgtagggcaggccgatgttgcagacgccgccaggcgtggccaggccgatcttgccgccggtcacggtgtacgggccggccaccgcggcatcctgcagcagcacgacgcgcttgccttccaggtgccacaggttgtcgatggtgtcgcgctgtaacgtccagctggccagcggcacgccgcgcagcgacgccggcaccgtgccgatgctgcgcgccacgacgtgggtggcgtccacgtaggaatcgatcaccagccgcaccttgacgcgcgtggtgctggcgatgccgtcttccaccgtggtcacgtcgcgccacagttcgaagccgtcaccgacatccgtggcgccgacgaacagcgcggcggaagcggtgatggtcagttcgtcctgttcggtccagccggcggtgctgcccagctggatcgtggtggcggtcgcgttccggccgtcgtactgcacaccgcagtccacgaaccacagatccgattcgctgttcgcgcgggtcggcgcctgctgttcgatgcactgcaccacttcgccgtcgatcaaccgttccaccaggaaatagcattccgactccttcttgcccggcagcgcgcaggcgtccaggaacaggccatcggtgtcgtgccagtgccagcccacgacctcctgttccggcatgtacgtgcagccgatgcgcacgccgtcgtcgcgggtgaaccacaccacttgccagggcgccttccagtattcgatccactggacttcgaagccggcgaacaggtgatcggcccacacgctgatgtcgttgccgcggaacccgtccttttcgaactggtagcgcagatcgcggatcttctggccctcttcctggatgaagatggccgactcgccaatcagcttggactgcacatcgccgctgccggcgttgccctggttcttgacgccgatggtgctgggcgtcaccacgtcgtcctgcccgcccgtgaccttgtattcgccgcccgtggtcatcaccagcaggttgtccagcggcaccaggtctttcaccgtgttgacctggcgcgcgttgatgacgaacgtaaccgtgtcgctgtccacaatgggcgaggaccggccgaagttggggtaatcgccgatgcacgacgcccaaatggtttggggatccgctggcgtgccggcgaaccacagccggtcggcgaagaactccacttccgagggatagccgtagcggcccgaccaggagccgaccgcccacacgtcggtgccgccctggccagcatcggccagttcgttaaccaggatgttgttcgtgccaaccggcggcgcttcgtagaaggtgatcgtgtccgcggtgggattgaccgtccagccctgtgccatcactgaatctcctgctggacgttggtgtttccgccggggcgcacgctgccgccaccgccgccattcacgccgccgccgccgccgtagtacgggttcggctggatcggctggccatcgatgttcaccttgtagtccagggtcgaaccgctcaacgcgcccgtgatgttgaacaccttggtgctgccgtcgccgctgaacgtccaggtgttggccggtgccggtgcggtgcccacgatgctgtccggcacacgttcgatcaccaccgcctgcacgtggcgcgcgtcggtgtaggtctgcacctgcaggatgccgaaggtgttgtgcaagaactcccattcgacgccgaccgcgtagctgttcacgccgtcgtccttgatgtcctgcggcccgtcgaaggcccggccgctgtcatggatcgggcgcacgttgccggcgacccagtagggcgtgcccttgccgcccaggctcggcgggatgctgacgcagcgatacaccttgctgtccgaccggcgcaacgcgcccacgggcacgttcttttcggcggacgcccagggcttcaccccgcgcagttccttttcctcgacgtacagcagcgaccccaccatgtcggcggtgaaggtgtccacgttcgtgctgaccgtgacgatgccggtggtgccggacaccgccatgatgagggcttcgtcgctgttgaacgggcggaacgggccgcgcttgaacgcgaagtcgcgcagttcgaactggttgaccgccaggcggcgcagttccttctgcggcacctggccgtggacgatgtagagaacgtccgccgactgggtgaagcgcacgctgcgcagcttcgcttcgtcgtagggcgtggccacttccacgatgcggtcggcgctgccgccgccggcataagcggtcaggatgctggaatcgaagccagccagctggaaggtgttggccgtggccaccgtcacggtgaaggtgcggccgtttaccttggtcatgccgcgcacgccggtaatcaccacctggtcgccggcaacgtagccgtgcccggtggacgtgaccacggcggggttcgcctggctgatcccttcgatgggcttctgcgcgttggtcagcagcgcgccgttgacccaaaagcggaaatacccgtcgcccatttcgatcaagtatttgacgctggtggagtagatgaagggcaccaggcgcgtcagcttgttggagaacttcacccggccgcggaagatcgtgccggggcgcttggcgccgccgccggtcggcttggtgatgaagttgcgggccatgcccaggctgatcgcgtagcgcgccagatcgacgcggccacgcataccgggcgaaagctcgccgccggacagggaaggctgcaggaacttgggcatgtcagtacggcccccggcccggccacacgttgctgtcgcgcgcggccagggccggcgtcacgtagtcggcgtccgtccgcgattcgttcatggcgtgcgcgcccgcgttggtcagcgccagggtgtattcctgcagcagctgggtcttgttgttcaagcccacttcgccgatcaagggcggcgcggcttcggcggcgatgcggcacgccagggcgttgacgaactgcggcggataccggccggtgtcttcgacgcggcaggcgtacaccaggaaggcgttgcgcacgttcgtgttgatcgtggtggcctggtcgccgtagctggtgtcccagtcgaaggcgccggatccccacacgctggcgatgtagtcgccgttcgtgaagcgggacagcttgccggcggcggcgatgccgttggcgtccgtgaccgcgtaggcggtcaggcaatcgttcgggtacgcatagcggtagtaccagcccggttgtgcggcttccacgtccagggccagcgcctgcgagcgcacagcccagggccacacccgttcggtcagcaccaggtcgcgcatcggctcccacaggcggttcatcacgtcggcggccttggattcgtccgtgaccgccgggatggcgatggactgggccagcttgtagagcgccaggttaaaaatgtcggtctgcgtggccacggtcatcacctaaaaagaggggccggcaatacgccgaccccgactgcacgcccgccggggaggcgggaattacttggccttgtcgccggtcttcgcgtcgcccttggccttgtcggcttccgcggctgcggcgttgaccttttccagctgcgactgcgcggcggccagttcctggcgcgaggcttccagctgggcctgcagttcgtccgcgcgctgcttctcggcggtcgcctggtcggccgcggcctgggccttggcatcggacgccgccagcttggcgatggcatccgcttcggcctgggccttcgcctgggcatcggcagcggcctgcgcctgggtcgcctggtcggcggcctgcttgcggctcacgtcctcgctgttggccttcgccttgatcttggcggcggccagcacggcaaggcgctgggcgtcggactcgctggcggcggccttctcggcatcctccggggcgacttcgacgtaccagcggcccggcgtgacgcccggtgccagcgtgacgatggcgccagcgccgaccaggccgtaaccgtccacgtagtgctgcggcgcgccgtgggcgatgacgtactgctgttccccgcctgccggcgtgcgtgccgtccgcgggttcagtgctttggtgttgctcatggtgcagttccttggtcagtggaaccggccccgtagggccggatccagggcggtcagttgcgggcctgggggttgttggccgccatcttgcgccagtagccgggggtctgcgtcaggaaggcgcggatggtgccggcggtgccggtcccggtgatgtcgtagatgaggcccacgtaccgttcgtaatcgcccggcggcaccggcaggaccgccaccaccttgttcgcgcccaggttggccaccggaatggcgcccgtggaagcgtgggtggtcggcgacgtggccaggtcggcggtgctgtccgaagccagcttcacttccagcgcggtggcacccgtgaacgcggtgccggtctgcacgaccaggaacaggtcgccagcgaagccgggggagaagttggccaggaccggcgcggtggaaccgcggtcgatgacattggaaatgccatcggcaagcaccgcctggttgtcggagaagtacagcagctgatcgaggatcatggtttcgattccttgtgaatggccggcgccgtcgattagacgacgacgcgggtttcgttgagggaaatggcgtccatacgacggaccggcacgccatcgaagtccgtgaccttcttgcccgcgatttcgcgggtggacagccacacgttcgccttgttctggatctgcaggcgcatgaaggtgctgaccacgcgcggcacatagaacaccgggttcaggccgttggggttgttcagctgttccagggccatggtcatcaggttgatgagcttggcgcccgcggtgatcccggtgatggggtcgccggcctgcaggtccgaaacgtcgatgttggcgatgcggacgatgttgcggtaatcgctgacggcgataccggcattcaggtcgaaccagtcttcgaagcccaggtacttgccgcccgtgccgtcatcgatcatcgcctgcggcagcgggacgtgcttgatgccggcggtggtgcccttcgggtagaagcccatcaccgagccttcgccccagccgaccaggtagatgctggtcaggtcggcgccggtaccgcccgcgtcgatgatctgcaccgcggtgcggtcggcggcggccaggctggcgtagcgcggcgcgatgcccaggaagtcttccggcaccacgttcggatcgccgtacagcatggactggaagaaacgctggcccatcgattcgatgtggcccttgttttcgatgaagcggaaacgggccttgtccacggccagttcgaccagcttggcatcgacctggcccagggcattgaacaggccagccgattccagcacggagccgtaaccggacttcgacgggcggatgccctgattgatgcggcgcaggaaggtttccggcagcttctggcgggccgacaccttgtggccggtggtgctgttggcctcttcccacgggatgtcgttgaaagccgggttggtctgttccagcagttccgcgatggtgacagcggcgccggaatcagtggtcagggccgccgcatccgcaagggtgggctggccgttggcgagaattgccatggtgcgattcctttttcaggtggtcaggtcagggttgagggcattacatgtcggggtacatgcggttccacggcttcacgtccggcttcgcggccccaccattgccgatgccatcgacaggcgaatcccgcatcatcttgccgaacattgcgaaggccttgataagttccgggtggttgccccagcccaggttatcgaacgcctccaccagcttcgggttctgcagcgcgtgaaccgccgtggtggcgaatttcacttcggcgtcgtactggtcgcccagttcggctttcgcctgcttaccccattcgtcgcgctgctgcgccacagcggcttccatggcctgctgctgcaccgcggcgtcctcgcccaccgtcttgatgaagtggtcgatggcccgctgcgctcccgcctgggacaggcccaggtcacggaacagcgacagcgccacgtccttccgctcgccttccagctggaagccgtccggcagggtgaagtccgtgtacgcttcgggcgcgccagtcagtacaggcggttcgtcgtcggtcttgccctggccgtcgccagtcttcccttcgtcgcccgtcttgccctggtcgccctgcttgccggcgtcgtcgccggtcttctcgccaccctcgccctgacctcccgaaacagccggcgcgctggcctgctgcccgttcgggttcgctgcatcggtggctgcacctgcgccgtcgccaggattgggttgctggccggcggcgttgttggtgtcttcggtactcattgttcggattcctcttcggtgggtttcggcttggactgcgccaggccttcccggcggatctgcgcttccttctccgggcagtggtcgcgcaccaggttcagccaccacttcgccgcgtcctgcatcccgattgcgtgggactgcgccatggcgttggtggcaaacggtgaagcgtccagcccggtctgcagcatgaacagccacaggatacgacgggcggccggcatattcatcacctgctgcacgtcggcccgcagctgttcctggaaccacttttcggcctggcgggcttcgcgctgctgggcttcgatggcatcgcggtcggcggggtgcgtcatgcgaacccccaccagcacaggccaccgacgatccaacaggccgcggcggcgacgccccacacgatcaccccggcgccttccaggtcgagcttacggcggcggtcggcggtcatgctgcctgtcccccgcgcagctgttcggccaggccttcgcccaggctccccggctgcggcaccgcttcgttcagcgtcttgatcgcctgggcgccatcggccatcggcttggccgcagccagcgccgcctgctgcgcttcctgcgcggcgcgaccctggcggatggccagcacggcgtcgtcgtcgcggacgatgctggccggcgcgcccgtgcgctcgctgtattcgtccaccgcctggtcggcgtcgaacttgtccagggcggacgggccgaacacgctggccatctgcgcgacgaacccggcggtgcgttcgatgccgctggtgcccgacgccttcatggcctgggccaggatgctggtgtattcgatcttcaaggggatgctggccagcacagccggcggcggcgggatcaagccggcgcgctcgcacaggcggaacacgcgcaccacggtcgggtccaggccttcgtcggtgacgatttccagggtcggccccagcacggtcgccttctcttccttgcgctcggcgatttccgtggccgtgcggccggcggcctcgcccagggattccagcatcaggaacaggttgtaatagaacgaatcttcgatccggctttcgacctcgcggatttcctgctgcacccactgcagcgaccccggctgcggggtgtaggtggcttcgatcttcgcgctgttctgattctgcggcaggtagttcttcgtccgcggcgccaggctggccccgatgttgcgcatggtgtcgggcacgctgaccggcggttccgccatcaagtcaatcaggcgcagcttctgcccttccaggtactgcagctgtttgatgtcgcccagcgagtcggtgccggggcacgcggaatagctttcgtcgcccaccgggttgaagcggatgcacacgaacggcggttcgtagtggccgccgatgtccagcacgccgtgcttttcgtcgccgctgccgctgatccacaccacttcgcggaacgggcggaacttcggcgcctggacgcccagcggccccatgccagggcgcgcgtcggggttcggctcgtacagggcttccacggtgaaccgctggtccgggctgcgcttgtacgcctggatcacgcgctggggcagcttcgcttcgtcgggcacgcgctcgcccgtctccgggtccatgcggccgtacttctgcaccagctggcgcgcggtcttcgtgtagcagcgccacagcgaatcgaccttgccggcgtcgtccagggcgatggcatagctgccgatggtcagcgggtggaagcgcacgacctcttcggcgttctccacgatcatcatggccgccacgccgtaggacaggtcttcggtgtagcagaccggcatggccttgtagaaattcgacttggccagggtgtcgcgcaggatggtggtcacgttgtccagccacacgcgcacgtcctgcagctggcccatggccgggtccggcgtggtcaggttgaaccagggtcgggccttgctggtcatgtgcgaggacatgccggcggtggccacgcgcacgcacttggtcgcggtgccgttgatgatcttcgaccggctgcgcttcttcgtggtggtgttggtgccctcaccgttgaaccggccgcgggccgggtcgatgtactccgtcacctgcatccagtcgggcatccatgcttcgcggtcggcgatcatcgcgccccggcgccggtcgcagtgctggcgcagctgcagcgtcggctgggccgcggcggcgtcgagcttggcgcgggcggtttcgatgtccatggcttcccctgtcagatgccgaaggggcgcagatcatgcgccccctgctgcaccaggatggaacggatggcccacggcagtgcagcgaccagggggcgggcaaggtattggcgggtggtcttcatcggtcgggatcccagcacggtcttcggggcggcgaactgctgctgcgcggccagctgctgctgatagttcgcggcggcggcgcggcgctccgggccaccgttgcgcacgtcctggcgcacgcgctccgtctcggcgttgcggcgcagctggccggtcgggtcgcccaccgcggtcttcgtcaggccagcaggatcggcccagcgcgcgctgttgccggtcaggagcttggccgggtccatcaccttccccatggtggtcgaattgcacatgcgtcagacccccagggcagtcttcacgggtgcggtgggggccgtgccggtgttgccggccaggatcgtggactggcgcccgccgcggctgcggatccggttgcgctcgcggtcgcgctcggcgacagcggcatcatccacggattcggggccgaccacgggggccgatgctacgggcttcactttcggggcgctgctgcacatggtggtcagtccttcatcacgggatcgtccgcgtacatcgcggcgtatttgctggtcccggccgcggccagggccaggtcggtgatctgcagttccaggcgccggctggtcttgccgccgtccaccgtctcttccccgaccgaatacaccagggcaacgccttccagcgccaccttcgcgccggccaccggcagggacttgatgcccagggcgtccagctgttcttcggccaggttgatccgcagaccccacgggaagtcgggatgctcaccatgcacggtgtcgcagcactccgcgtccttcgtcttctcttccggcttgcgcttcatcgataccagtttcatggcgtcatcccagtgggttgtagggggtgccgggctgaccggacccatacgattcggccacctgcgcagccagcgactggatgcgagggtggccgatgttctcctggctccggtcccctggcgccacgtcgaaagcatacgtcagcgccgcggcgtccgcacgatccggcgagtggcccagttcttccttcacctggtccttctccaccacgcgcatcttgtcgccctggaaatagtaggtgtgggcggtcagttcgcgggacaggtcggggtcattgggcaggcacaggccgtcgtgcttgatggcgtgggccagccggaaatacatttcggtgcgcttgttgaagtagcgcggatcgtcggccttgccggcgaagcccaccccggtcacggtgtagttcagcgcgcgcagctggtcgatccagccggcgccccagccgcccgtgtcgtccacgaacaccgcgtctggcttggcgttggtctgatccttgtagaagtcgcgggcgtcctgggccacccagccggcgccctgcaggctttccatgttccggccgatttccagggggaacatcacattgccgttgcggcgggccttgcagctggcgtcgtcgccgaaccgggccacgtccacgccgatgatgcgggccagggcacgccacgactggtcggtgggctggcgcttcatggccgcggccacgtcgtccggtcccagcagggcgttcatgctggacggcgggaacttgccgaagacgttgaccagcacccacgggttgtcgcggccgtacttctcgatctgctggcgcgcccactcggcggacacgcgcggcgtgcgcttcgggtcatccgggtccgacgtgatttccaccagccaccacagatggcgttcgctggtggtcgcccggtacagcggcccggacaggtgcgtggggttgcccgccatcaccaggtgcgcgtgcaagttgatcccgtccgcgttggccaggccggcttcggccgcggccatcaccgcgtcggggatgccgccggcctcatcgatgatgaacatgatgttgtcggcgtgcaggcccgccagggtgtcggcctgctgttcggtgctgccgcccttggcccacgaccggaaggacatgaaccaggtttcggggttcgcgttctcgtaaatccgggtcttcgtccaggtgaaggtcgcctgcagcagcggcgcgcgcttctgccacttggacatttccgaccacaggccgtccgccaggttgtcggcggtgatcgacacggccgcgatcttcgggtgcatgtagcacagcaggaagttccagcacagccaggccagcacagcggtcttgcccggccccttacacgccttcatggccaggcgcgggttgtgcgggaaggccgccagcacgtcgtcctgccattcgtcgggggtggtgccgaacagttcccggaccatctgccccggatgctcgcgccagcggcggatgcgctggccggccgtctccgggaccggggtggtgctgatgccggtgtcgtcggtcacagcagcggttcccccgaatagtcgcaccagcagcgccgggcgcgcgcccagtgccccatgaaggactgcaccggcacggtctgcgggtcagcgtagaagccgaccgcggcctggtcgaaggcctgggccttcacgcgcagttcgtggtcggccggcaggccatcggcgtcagccctggccaccattcgccgggtcagttccgcgctggcgttcaatggccacccccgccggtaccggacccgcccaggctttccgcgaccagctgttccagggtcacggcggccttcacttcgaccttctggccgtaggtgcgcggcttccgcttctccatgcgccacctcatgttcgaaagcacgacgttcgcggccttcgggtccagcggcttttcaccaggctgcagatccaggcccagcacctggcgttcgatgcgctccatttcgtcgtagtcggcgtccgctgcagcctcgcacgcgcgcacgcacctggcgtcaaagtcggcatcgtcggcacgccagcggcgaatcgtggcggtcgagggaaggccggcagcgtcggggtcggtcgagtcgaaccaccggaaggacttgccttcctgcagcaggcgcacgatccggtcatccagatccgagtgccggacggtcgggcggccagccatcaccacacccccatgccgcgttcggtcatccacagggcgccgatgatccccagcagcgcaatgccaggaccgccaccggacggccccagccatgcacctgccaccagggagccggtgcccagcaccagcccgcccatgacccagcccgtggcgcgcagcagtcgcatcaacgcatcccgagccagaagcaggcggccgatgccaccaggcaggcgatggccaccagctggaacacctggccgaacccttccgccttgtcggcgatgccctggtacgcggtcaggcccggcgtcaccagcagctgctgttcggcgatagccgcggccgtgtagttgtgctgtgcccagtagctggcggcagcggcgacgatggccagcaggacgccggacacgtgccactggctgttcgtgaacaccagcaccaccaggttcgcaaggaaggcgccgacgatcaccaggatggcgaaggcgatggtggcgagaaacgacaggttcatgggatacgctccgataacgatggggtaacgatgcaggtaacgcttcgtgcgttacttcttccgtttgatggccggcgacggggtgcccagcttcggcaccggcttcccctggacccgctggatggcgtccaggttcgattcgtagaactgcaggcacttcttccgctcgcgggccacgctgggcatgacttccagcggcgccgtctcccgccactcgcacttcgcggtcaggtccgggtcgatgggaacgaacacctgcacgggcacttcgacaatcccggccggcgtggtcgggatgtcgggcttgatgacctggcgaccgcacgcggccagcaggatggacgggagccagagcagcgcgcgcatgtcagtagtccttcaaggtcgggcaggctgcagccatcacttccagcgccgccttgcattcgggcgggcgctgcaggaaggcgtcctggtacttctgttccgactcggcggccagcgcctgggcggccttcgccgcggccagggcggtcgcgttgtcccgtgcggcctgttccagcagcagcttctgctggcgggccaggtccgtgaaccgggcgatggtcgcttcccgatccgcgatctgctgggccagcgtgcgcttctcctggtccgtcgtctctttcaggcgggtgtagtcggcccgctgctggacgatgaccgtgccgcgctgccaggactgcaggccggcggccaggaacagcagcgcgaagaaggcgcaggcgccgcgggtcttgttgcccggttgccgcagccacttccgcgccgtctcggccgcatcgcccagggcgcccaggatcgaccggaccaccttgaccacgccgcccaggcccatgaagtacaaggccgccacggcgatgatcgccacgacggatccgccaccaacccaccacagccagttcatcggtcattctcccggcggcgccacggtgccagaagcagcacagccagcccgcacttcaataccacgatgtggaacggcggcacctggtggccggcccactggtcgcccaggatgaccagcatggggatgccgatgcacagatgaaccaccagccacagcagccactggccgatgcagccgaacgtgtgatcggtcggccggcgcgtctcgtacaggcgccagcagaccgcggagaacaccccgaaggtggcgcaaaggttgaccaggtacaggatcacgggtcgcccccgatgacacgatccgcccggcgctccacggctttcagcaggccagggagccacggacggatgccgacgcccaccaggccggtgacgggcagcaccagggattcgtccaccaccaggcgggtcagcgtcttgacgaacgcgatgccggcctggacggaccaggcggcgatgaaggagtaagccagcacgacggcgcccaggaagcccgcggtgaacagcaggtacagcaggcgacggcgcaggctggaaccggggtcagtgctgatgcgcgcggcttctttcgccggaagcagaaacacgccgatcatggtgccggcgatggccacgtacagcatcgaaatggggacgttcaggaaggcggtttcggtcttcgtgacgacttcacccacggcgccaccagcggacaccacggccatcgtcaacgctccgattttccccatgcccatgtcgtccaccgtcaacctgcccgaaggtacaggctacgttccgcggcgcgacggcgcgtgaggcccgccattacctggccgccggccttgttccagaccgggaactggtcagccgcgcaggtgtggcacccttccatggccttgcgccacatggtcgaggggcggccggatttcagcatgaacagtccgtccttgcccggatccttgccggcggccttgcggccctcgccgacgttgaacaggaagctggccagggccgccacctgggcgtcctgcagcacgccgccgtccttcttggcgcgggtgcgcacggcgttcacgcgcagctgcacttcctcttccaggttggcgcgggccacggcatcggaccagggcgcggtgtcgggggtaatgaactttcccgtttgcccgtagccgatagtccagggcgcgccggacagcgccgcagtggcagccggcaggcggttcaagatcgaacgggcggggacgtggccccagggttccttccgcgtggccttggccaacgggctggcggggtcgggatacggatgcgggcggaacccttcgaactcggcgacgatgggcagcgcgagcttcgcggcttggtcggacacaatttccccctggacacggtttcgcggacggtggcgtgatgatgggccgcgcgccgtgggcagtcaatgaaaagccccggctgctggggaggcagaccggggcggggaggcggcagaggatggccgccggaacagcgttgcacgtcaggcgcgggcggtcaatcgctccgctcgggcttgatctttgccacctttcggcaagcatccagccttgactgcagccgcctggcctggtgcagcgcatcaccgtcgccgcgcctggctgcgcgatgaagctgggccaggcgcggcgcgttgtaggcaacgaacagttcgcggtccagttcgcccaggctggccgcccactcgcggttcgcctgcgcgttgcgcttagaccgtgctgacatacggatgcacctggatcaccgcgccaggcctgcgcagcgcgtcagggtgcgcgcccagggtgtcggcgggataggtcttgatcgcccggcactccaccacgcgcgcgtcgtccttccacacgccggccgcggtcagcgcgtcttcggtgctgcgcaccagtttcgacaggtcgggcagctttgacggatacgatgcgcgccgcttgggcagcgacagcggcgccggcagcgtgaacaccaccagcagcagcagcgggccatccatcggcacccagtcgcctggatcctcgcgccgtccgatttcagcttccgccgccaccttcacgtcctggcgccagggcgccacgcgcttcgatgattcggccagcaccgcgtgcccgccgtggatgcccttgaaggacttactgccctgcggcgccgggtcgccgtacaccacgatcttcatgccagttccctggcagcgcgcgcgtcgaacttcaacacgcccaggcggatggcttccagcagcgtggccttcaccatgtccgcttcggtcttgccgtacttctccacgaacgcggccatgccggcgtgcagttcgcggtgttcctcatccgtcagcggcatggtgtcgaagtcgctgaccttgtgctgcgacagccggccaccgatgcggtggtgtgccacgcagccgatcatgccgctggccgcggacggcagcgaacggacgaacgccaagtattccggcgcttccttggggagctttgcatacaggtcgcggatcattttctttcgccttcgggttttgtgagcctggccagttcgaccaaccagtgcgccaatttttcgggggtatgttcgcgctccgctttcgaaacttccgggcgccacttcggatggcctttcttcattcttgatccatcgcgcagcgttctgttttgcgcaataacatgggtggaccctcccagcacaaaatgcatagcggggacatcctgcggttcgatcccgcacacgtacagccaggtcgccttttcggcgcgatggccgaaccagtgctgcaggatcgggatcgtaaatcctccccagctgtcccgcccagcacctggcaacggaaggccttgatgcgcccaaagcgttgacgttgccgggtgttcaagcaccccccccagcgacgaaccgcagctaccgcaaacacagccaggtcgcgttctccttccctgggcttggccaccatgcgaagccttccccaggaccggcacggcggatgcgctacaacaggcgcgccgccgtcccacgatctggcatccctgtcgatgtcataaacatcacacccggatattttcttgtagatgctgtcctgcctggcgaaaagaacggcaacggtcatggttgctccagtagggattcgaagtctgcgacctgctcgggcgacaggtcggggtagtcgtgttcggcgacgtattcggtcatcaccttgaaagcggcggcgaattcgtcttcgtccatttcatcgaaggaaatgctgcgcggctcgctgcgtgttacccgggtcatgcccatcccagggatgtcgatgtcgtaggcgatgcgttcgcaggcggcgccgctgcgcgcctgcacgtccttcaccgcggcgtgagaatccggcttgcccttgtgcgtcaggtggtggccgtagccgtccacgtgcgtgaccaggaacgtgccgaactgatgcaccaggcggtggaacccctcattgcgcgggttcttgatttcgcagcgcacgcgcccatcggggcggaacttccgcccctgcaggatccgccgatccacgttgctgctggccaccagcgcgcgcacttcctcgccggtcgccgggtcgatcatcgtgcgccacttcatgtagacgtagcgccgcgcgatcttgcgcgtggtcgaatgcggatggtcagccattgggatacccgtcatgcagcacgccgtccagggtccggccagcggcgtgctttccgaccatgaccatgcggtgcgcgcctacgtcctgcgggacgacatcgtgcccgcactgactgccgtcacgcatcaccgccatctgccgaacagggccgcaggcccacaggtcgcgcggctcccactcgccccactgcttgaacaggaacggcacgcggtatgcggcgcactggtcgcgcaacatgcgcgcccaatcaggatgcagaggcctggcgccacgcccgctttcgccaccgacaatcacccaatccaggccatacaacagcggcggatcggtgggctggccgccacatccgcattcgtgcccgctgcagcacatcgccggcccgttcgggaacaggctttcggggtaggccagatccacttcgcccagcagcggttccatcgacaggaacttgaccgccgcgcgtgtggccagcagcttcggaatgtcgcggtcggcttcggcctggttgcagatcgtcgcgcccagccacacgttcgccggccacccgccatggatgttcgccgggtccgggccgtgctggaccgggccgccgacccagggggcgggcgccatcttcgccacgttgccgatgcgcttggtcagcagcagccagtccaggttcggcgtggcttctatcaacgcgaacaggtcggcgcgccacgccgggtccacttcgttgtcgaacacgtcggccaggctcgcgcagaacacgcggcggcgccggccgttctccgagaagaactgatcgtgctgcgcgttccaccgcagcggcagctgccagttcgaaggcgcggtgcggcggcgttcctcgcctgcgccccacttcacgccgaaccggcgcgtgggcgtggacacgctggcgtagcagtggtcacacgccgggctgattttggtgcagccgatccacggattgaacgtggcgtcggtccattcgatcttgctttcgattgccatggtgttcccctctctcccgttggttattggccgctggcgcgccgctcggcggccagggcttcgaagtcacgcatttccgaatcgctcatgccctcgcggcgctggaacgccgccctggcttcctcgctggccacgtccccgaagtaggtgcgcaccagcggcggcgccggggtatcagcgtccaggctcacgcccagcagcaaacggctgaccacttcggcaggcggcagtcggtgccgaaacgccaggatgcgcagctgttccgcagcgtccgccgtgatgcgtggcccgcgcacccagccttcggccttcttcttcgcttcataccgctggttatgctcgcgcgctgccatcactgccccctgtacttttcggtcgcctcgcccatgagccggcgcatttccgtgtcggcctcttcgccttcgccataggcgccgatgctgcgctgctggcggatgaacgccagggcgttttccagcttcgattccgacttcgccagcgcggccttcgcgccgaacgattccggcggcggtgccggcgccgtggccaccttgtccttcttcggttcgtcttcccaccgctcgccgttgatgtaggtgctgccgtgcgggatgaagccgcgcagccaatcgtcgtcctcgcgctccatgcggcgcacgtgggcaatgatctgatccgccatggcatcgcagcctttcagcttccactttttcagcgcgtcagccttgcccttcttgaccgggtacgcggcccaaaacttcgggaagtgttcggcggtctgcttcttgccggtgccggtgatgcgcttgggcggcggttgctcgccttcgttatcgggcggtaccggcgcttccggcttcgggatgtccttgggcaattcgtcccgcggcgcgtcgtcgtggccagcctgctggccggtggcctttggctctttagaatcttcttttctcttctcttctttaggtaacgcaccactaacgccgccagcgttaccgccatcgttacctttcgccttgtgcttctgcactcgtttggccgtcagggcgcgctgcttggcggtttccccgttgtgccggtcgaagtgaggcagcgacacgcccgacgcatcgatgatcgcccaccgctccaccgccatcgcggcgatgaacccaggaacgccagcgacacgatcaagcaacgatgaagtaacgcgcgcagcgttaccgtccacggtgtgcgagtcgaaccacgaccacacccgcatcagctttccgatcaccgcatccgggtcgatgcccagggcttccgcgatggcgaacacttccggcttgtccagcgtgtccttttcgaatttcagccagtcccctgccatgtcacaccgccttccaggccgcaacgtgggcgcaatggcagtgcgcggcgcgcgactccacaatgcccacctttgcaatcagcccggcccgtgcagcgcgctggaacaccgaaccccaggcccgcagatgcggcggcgccggcacggccgcggcggcaatgctgctgcgcacgtcctcgctggtgaaggtggcgccgctgctacgcttgcccgccgcgaagatgcgcagggcttcgtaggccgtgtccccccagttcgggttcacgtcttcggcatgatcggcggcctgctggatcccggcatcgcgcgccgcccgcgcggccgtccaatcgaattcaggctggttcatgtggtcgctgccttgcgccgttcgcgctgcacgatctggctgacccgctgcctggtgatgtccaggtcgcgggcgatttcggcgatgctgtcgcccccttccacgcgcgccatgatggccacgatgcgttcccgctgggccttctgcgccgcggtctgcgccctgttccacgtcttcgttttcatgtcggggtcatgccctgttcctggttggtgacggcgccaccttacccccgcaacaggaattgcgcaacaggggttgacaacttccgggaacggcgtatcgttggcggcacaaacgagctacggccaccgagggatcccatgcgcatcaccgaaaagaccagtccgcaaggcgtcgccatcgaatacgtggagcctgaccaggccaccagcgaacgcgacatccagcacttccgcaccatgatcgaactgggccgggagaagcaaaaccgccgcgacgcgaagcgcccgcagcaggccgccgtccaggaaggtgccgaatgaaccactgccccgtcaccgcagacctgaaccgccacctggacgaactggaccgggccgactcgcgcagcgaatgcgtggacgccaagctggacgaactcatggaggacgcggccgaggttggcagcgccctggacatcatcatgggcgacagcgacgtgggcagcggcggcaacaccctgttcgctggcgacctggccgcggtgctgctggcgtccgatgtcgccttcggttccgaggccgtccagttcttccacaagctgcgcgagcgcgtccgcgaccagctgcgcagcgacgccgaaaccctggtggatgaagccctggccgaatccgaagacgccgcggcggaagcgcgctacgaagcccagcaggccgaccgcgaacaggggtggtactgatgcgcgcccgcggcatgttcctgggcgcgctgttcgccttctccggccccgccctggtggcggccttcttcatggacaccctggtgccgcttgtcatctggctggcggccaccgcggtggtgatcgcgtgcggacgggaggcatgatcgtggccagcgaagcgaagtggcccagctacctgggcaagccggcggatccgctggaaaacgtggtgcgcacgcgcgcccagtccatcctgacggaagtgggcgcggtcggcccgcctctcccctatgaccaggcgcgcgatgtcgtgcgctggcacgaatcgcacctgcggagactgcagggcgtcagcctgggccaccggctccggcagttgttccacctttccaccaacgacaaaggaacgcagcaatgaacccgaaccacaccagcatcgaaaccctgatggccgaactggatggcggcaccctggggccgcgcctggccgccgcgctcgccgaatccgccctgggcgtcgccgcctgcaacaccaagaccaagaagggcaaggtgacgctggaattcaccatcaccccggtgggcggcgatcagacccaggtgcagatcgaccacaccgtgaagttctcttcgccgacccagcgcggcaagaagcaggaggacatttccaccagcagcgtgatgtacgtcagcaaccgcggcgccatcaccgtgctgccgaacacgaacaaggatctgttcaagcccgaagaaggcgtgaccggcgccaacgtcgccgcgatccgctgatccccaccactcccgtttcatccaccgcaacaccaacaacaggaaaccgaaccacatggacaagagcgcaatcgaagcgatccaggattccagcgccgccgcggccaaggccacccaggaacagatcccggccagcatcgcgcacctggtcgccgtccccaacggcgtcaccctgcagaacgtggaagcccagctggccggccgcacccgcttccgcggcaagctgaccaccagcagcatcccggacttcgttacctacgtgaaggcacgcgaaggtggccacggcttcatcgacaccgacaagctgggcgccaccgtgttcttcaacctgggcgacgccgctgcgccgggccacgccgaccacaccgcccgcctgaccctgcaggcgacccccgcctacctggccatgctcgccgctggcggcaaggcgttcagccagcgcgatgccctggacttcatcgaagactggtcccacctgatcggtgcgcaccaggtcagcgacgacggggcgttcaccccgatcccgctggcccgcgccatcgcggccatccgcaaagtgaagatcaaggcggaatcgaccaccgagcagaccgaaggcaacttccagcagtcgcgcagcgtcctggaatcggtggccgcgtcgagcgatgaaggcctgccggacgtgctttcgttcaagaccgaaccgtacctgggcctgccggaacgcaccttccacctgcgcgtgtcggtgtccaccaccggccgggaaccctcgctgcgcttccgcgtgatcgccctggaacaggaacaggacgaaatcgccaagcagttcaaggcgctgctgctgggcgaggttggcgattccgccagcatgaccatcggcaccttcgccccgtaacgggcgccacaccgcgcgacgcgcaccacagccggcgggccacccccgccggcactaccacaccaaggatcgaacgatgagccacgaaatcgacccggcggccgagcagaaccaggacgccaccgacatcgcaaccgccagcgccctggcgctgcgcactgccgccatgcaggaactggacaccgtggaagcgggcctgtccgaccttgccacgaaatacaagggcgtcgtgttcgacgtgaccaccacgaagggcatggacgaagccaaggccgcgcgcgccgccatccgcgaaccgcgctacaaggccgagaacatccgcaaggaaaagaccagccagctgtccaagctgggcaaggaaatcaacgaacgcgccggcacgatcaaggacgccatcctggccatcgaagaccccatcgataagcagatcaaggccgaagaggaccggaaggaagccgagcgcgaagccaagcgccaggccgaggccgaccgcatcgccggcatgaacgcgcgcctggacaacatccgcaacatgccgctgcaggcggtgggcgccagcgccgacgaactgcagcaggccatcgaccgcgtggccaccgacgaactggaaggcttcgatgaagtctacctgccgaccgcccagcagacccgcgacaccgccctggacgccctgcgcaagatgctggccgagcgccaggcgctggacgaacaggccgcccagctggaacgccagcgccaggaacaggccgcgcgtgacgccgaagccgccgagcagcgccgcatcgcagacgaagccgcccaggccgagcgcgaccgcctggccgccgaggcgcaggccaaggccgacgccgaagccaaggcgcgccgcgagcagcaggagaaggaggacgccgaccgtgccgcccgccaggccgaggaagaccgccagcgcgccgcgcaggccgaagccgaccgggtggagcgcgagcgcgtccaggccgagcaggcggcgcgtcaggccgaactggaccgccaggcggcagagcagcgccagcgggacgaagccgccgcccaggcgcagcgggaagcccaggagaaggccgaccaggaacgccgcgaccgtgaggccgccgaacaggccgccgccgcgcaggcgcgcgcacaggccgaagccgaggcatcccgccgggctgcgctgctgtacgtggtggccatgccggacggaagccgctgggcggtgccgctgatggtcattgcgaccgaccgcgcgaagcactacgcccaggagttcgacggcgacctggaacgctccctggccgaagacaccctgccgctgttcgacgccgacccgtaccaggcccacgactgggcggccaataacatgaactggtccgacgtgaagggcgaagcccggatctacgagccggccaagccgctgggcgatgacgacttcgccgaaggctgggtgaacggcgaataccaggtggtcaacacccaggggccgcgggcatgagcatccagggctggtactacctgcacacgaacggcgaactgatcttcaagccgaaccccgacgcggcgtgcgacatccgggattccgacttcgcccgccacctttggccgatggaccccagcgaccgcgaaggcgcgtggaacatcctggtggaagcgcacgccctgggcgcgcaccaggcgcgcatcgatgacctggccgcgaagtggggatgcgacgacgccgatgccgacaactacgcccagcgcgtcggcgtcaccatccagcgcgacggcgatgcctggtgcgccaccggccccggcttccaggacatccaggcatccccggtcggcttcggcgaaaccaagctggaagcgatggccaacctggcgcgcgcactcggcatgtccgccgggaaaatgtgggcgccgaccttccgcgatcttctgaaaaaggcagcatgaccatgaccaccgaaaccaacaccatcgaaggcgaagtgctggacgccatgccagccgcacagccggcgccgtccaccgcgctgacccacgccaccaaccccttccagcagatggccgtgattgccatggagaagggcgccatggatcaattcgaaaagctgctggatctgcaactgaaatgggacgccgagcaggcgcgcaaggcgttcgtggcggccatggcatcgttcaaggccgaacccatcgacatccgcaaaacgaaggccgtgggctacagcaccagcgacggcgggttcgtcggctacaagcacgccaccctggccgacgtggtggacggcgtggtggccgccctgggcaagcacggcctgtcccaccgctgggacgtgaagcaggaagccgggcagatcaccgtggcctgcatcgtggcccaccgcgacggccacagcgagtcggtcgaaatgttcgcggcgccggacaacagcggcaagaagaacgcgattcagcaggtggccagcaccgtcgcgtacctgcagcgttacaccctgatgtcggcgaccggcgtggccgcgaaggacatggacgacgacggaatcacgggaggcgcgccccaggtcgagttcatcaccgacgaacaggtggccatcctgcgcgacctgatcgacgcctacgtggtgaacgaaggcaagttcatggactggctgcgcggcgcgtgccgtaaccagcagatccaggcgctggaagaagtgccggccgattgctacaaccgcattcacgaccagctgggccggatccgcaagcagaaggtggccgagggcaaggcgcccgcagccgaaggatccaccaatgggtgacattgccgacatgatgctggacgggacgctgtgcgaagactgcggcgtctccctggacggcgaggcgccgggttatccgcggtactgcagcaagcggtgccgcaaggaccgcgaaccggctgtgccgaaagccacgaagatcccctgcccggcgtgcggtaagcgcgtcaaggcggcgggcctgcacgaccacatgcgcgacgcgcacaccaccaaggaaccgaccgatgcttgacgaactgcagattttcgaagacctggaacagggcacgcccgaatggcacgcggcgcgctgcggcgtcgtcaccgcttcggtctttcacaccgtgctggccaagggccgcggcggcgcgccgagcgagacgcgcaagaagctgctgtaccagctggcggccgagacgatcaccggggagtacgtgccgacctgggacggcaacaagcacaccgagcgcgggcacgtgatggaaccgcaggtgcgcgacctctacatggccaccagcgcgctggactgccgccaggtcgggttcatgcgtcgcggccggatcggctgcagcccggacaccctggtgggcgacgaaggcctgctggaaatcaagaccaagctgccgcacctgcagatcgaagccgtgctggcgggcaagctgcccagcgaccacgtggcccaggtgcagggccagctgctggtgtccggccggcagtggtgcgacttccgcagctactggccgggcctgccggaactgcgcgtgcgcgtgtaccgggatctgccctacctctccaccctgaaccaggaattgcagctgttcattcgtgaactggatgccctggtcgcacagatcaaggcaatggcatgaacatcgaaaacgacgtgcgcctgatcggcaacctgggcaacgacccggaagtgaagtacacgcagggcggaatggccatcacccgcgtttccctggccaccacgtcgaagcggaaggaccgcgacggcaaccaggtcgaggaaacccagtggcaccgcgtggtgttcttcgggaagctggccgagatagccggcgaatacctgcgcaagggttcgaagatcgccgtggccgggatgatccgttacggcaaatacgacaaggacggcgtgacccactacaccaccgacatcgcgtgcgaccagatgaagatgctggacgcccgccctgccgatggcgagcgcacccagcgccaggcaccgcagcgccagcccgcccagcagcagcgccaggcgccgcccatggacgacttcgccgacgacgacattcctttttgaggatccccagccatgaacgcagcacgtatgcagtcgatcatccatggcctaaccggcatcgcccggaaggtgtacgacacggtgccgatccaagaaggttggacgctggcgcaggtgtcggccgaactggggcgccacggcctggtgtacgaacacgcgaaggtgcatgggtgccttcgttcgttgaaggaataggggctgatccgcgaatgcgacggacagttccagcgcattgagcagcgcccgcgcctggtcgccgctcgcacccccaccgccacccaccaggaagacgacatgcccgcaccgaccagcagcgacccgatggccaacctggcagagattgccgccaccctgcgcgagcaggcgcgccagctgatggccaaggccgacgccctggacgcttcggccatcgaagtggcggaagccatcgaacgcagcggcgaggacggcgcgaagctgcgccagctgcaggcgctgctgaaagacatttcgaagtaacccgacccaccaccggccaaaggaggccagcaccatggaaagtaacgaaaccagtaacgcattcggtaacgctccgcgcgttaccaccgaacaggtggaggccgccatcatcggcgaaacctacaccgtcctgccgaacggccgcaccacggtctgtcagctgacgctggacaacgggttcaccgtcgaaggcctgtccgcgtgcgtgagcatcgaaaacttcaacgccgaactgggcaacaagtattcgcgccagcgcgccgttgaccaggtgtggcagctgctgggcttccgcctgcaggacacgctgccgcgcactgccggcggcctgccggaaggtggcgtgcgcgctgctgatgcaccgcccgtcgaacagttcgcgcgcagcgccgactgaccaccacggcgccgccagcacggggcgccactacctgcaggggataccgatgacacgcgatcaatggctggaaaaatgcgcggaacgcctgcgcgagaaggccggcatggaaccgggcgaggccgcggcctacgccatcatgctgcacgacaaccaggtgaacgataacgggcgcgagccgggcagctgggacgatcccaccgacaccgccgacgaagaaatcagctacatgtccgacgatgaggatggcgacgatgagccgtgaaaccagcatggaagcagccctggaacggttgctggaagtgatcgacacgccgccggcccgcaactgcgcgtgccacatttcgccgccatgcagtgactgtgtggactggggcggcctgcgcgaagccatcgccgacgcggaaactgccatggccatgcccgcggatccgatcacccccgaccaggtgaagcgcgccgcggcggccatagccaattcgcgcggcgggcgccggggcgtgccggccatcaccaacgtcctggacatcctgccgccgcacctgcttgcggaagtgaccgaggacgcgaaggccgcgctggaagccgcaggcggtgcgtcgtgaagcgccgccgccgcaccatcacccaggccgaggcccaggccttgaagcgtcgcgtggcgcagctggaaaacgacgaagagcgccgccgcgcagcatgggtatccggctacccggacggggtgaacatcgccacccacgacttccccagcagcgacagcgtggtgccgaccgcgctgcgcacggccaggaagctggggcacgccatcgtggcggtggacgatgggcacaggctgcggttctacgcgctgccgctgccgaaggcgtaacaggaaagggccggggatcacccggcccttctttcatggcggcgtcggccgcagccggaactgcaggcggttgccgcggttcatcccgatggccaccagcgtggcattgacgccactggccagcaggtgttcgatctggaaccgctcgcgctgcatcctgaaatacaggttgttcgcgcgaacgtaggccaggatcacgtccgaattcgaagagtagatggcgcgcttttcgtcggtggtcagccgcggcgtgatggcgccagtgaaagacgaaaagaccatggccgacacctgcgtgtcgtaccagtacagccacgccaccccgttctgcacgaacgccacgaagggccgcatgttctgatcgaacgccagcgccacttcgctgatgtccggccgcgagaagtacaggaacgccggcacggacggcgccgacagccacacgtccgtgcccagcacttccaccttccacagctgcacctgcagcccctgggctgcatcgttgatcgccaccccgcccatttcgtaatcaaccagcgggatggtccgccggctgacctgttccacgaaggcagaaggctgcggcaacgtcgaaagggaattgttggtgaacattacggcgtgtacctgccccagctaacggtgacggtgatggtcaattcctgggcgttcgtcttcgacaacgtggccggggaaatgctcatctgcgtagtgcatccaccgaacgcgaaaaatgccatgttggcgttcgtgatttccgtgcccaccggccacttcgcggtcgcggtgcgctggtacgtgccggcgacgtagttacccgaagagttccacagcccgtttatggtctgcgtggcgccggtaggttcaccagtgatcgcgccgaaggacgcgccggcataaagcctggtcggcagatactgcggattctgctgcatcacattgaacgggttttgcagcccccagccgccggtgaaaatgccgtaatccgaagtgacattcgcagcccgcatttcggtggtgtaggtggtggcgccgatggagaacgaaccggcgataccatccaggaacggatagttccgaagctcgtaggtcacgtccaagatttcatcggccagcacggtgatcgtggtggggttgccactgccgtcgcggataagagcgcgcgagaagagaaccgcgccggacgaaccccagcccacgccgacttcggaaaggttgccagcagcgacgccagcaccgaagcggtaagttttgcgaacccagccgtaatacggcgcgctgggctgcactccgctgggattggacaacgcggtggacgtggacgcaacctgcgacaccagctgcgtgtcgccattgctgggagccgtggaacccgacccaacaaggcaaaactggatgttgttgtaatggtagtccgttccgagccggtccagaccctggttcgtgatgaggttttcgaaccagtcggcaacaacgcgccggccgatttcctggccatccttgtcaatgcgcaccgcttcgatcttgtagaagccggcgacgccgtggtggagttcgatgttcatgcaagggttcccgaagtaggtgccatggtggtgcggatattctccgctgcgatggtgtgggtgatgagtacagttttcagggtgccgctggtggcggccatgatgggctgcacggactcggtaccgtaatcataggtccgctggatgtcccggagagtgccggaattggggtccatgctggcggttacgaagtcttccggcggcagggtgatcgccgactgcgtgttccgaatctcgccagccagcggcgccatagccgccgataccccgtcatcgaacacggggggcaatccgagcctggccaggtacacgccaggcatctgcgccatgatgctttcgaattcgaagtacgggtacggctgcgtggtcaggtaaatggcctgttcgcccacgcacccttcccacggcgcttcacggccagccgagtcgcgcacgcgcagcaccatgcaatagtcgtcgtcgctgttctggccggtcgggtaggagtggttccataccgccttgtctgcccacagacgccggttctgccgcttccggttggcgctgaccgccagggccacgtagaaggcgccagcgggcgcggaggcggtcacggtggaggcgtgccaggcgccgttactgcccgaccgcaccaggttgccgccgttccaggaatgcccctcgccgccgggcagcatgacgccataggcgtcgtaccaaatcagcaggatccgcgcgaccacgttgcccttgctggacgcgccctgctggatctgcacgctggcggtgatgctggtgccgacgatcaccggcaccttcgtcccttccaggctggcgatgccgcggccggtgtaggccgccgagtgggtgccgtcgtaggtgtcgaagccggatccgctgccgatgagccagcccgcgcccttcgaccactgcacgtcgccgtcttcgaaactgccattgggcaccacggtggtgtccgggtcgggaacctggtagccgggccaggccaccacgacttcgctggtgctgttgtccacgcgcacggtggtgcccggcggcatcgtgccggacagccattccacggtgcagtcgccgatgttgttgacgatctgcagcctgccttcgtaggcatcgccggccacgtacccttccagctggccatcgacgcgcaacgccggaagccccacgaatcgaagggccagcgggcgggtgaaaaggatgtggtggctggtcatggtcaggcctgcgccaggtcgccgctgatgatccaggtatcgccctctgcgtactcacacacgccggagataaccgaaccttccgtgcgcgtgtaaggcaggaacccggccgggatcaccagcgtgacatcggtatccgcaacgatgcgcgcctggccatcgccgcgctgcacgatgctgaaatagctgccgtccgccatgtcgtacagatcgccctgattcgcgcgcaaggtcagcaggcacgggttgacgttggtggtgcgcagcagcgcgaattcgctggacttgtccacggtgtaggtgatgccgtccacgtcgatgatcggaatgcgcagcgtctggaccggcgtggtgccggtgaacggcttggcgtagccgcgcaggatcacgaacccttcggcgccattcggcagcggcgccgggaagcgcaccgcgaagtcggatccgtccgatgccggcaccacggtgtattcgtcgtaaggctccttcgacaggccttccaccactacatcgtagaacagcaaatccgacacgtcggagccgggcagttcgaagtcggtatcctcgccgtcgcccgtgatttcccagtatttcgggctgacgccgaccacgccgccgccgttctggatctgttcgatgaccaggtaaagcgtgcgcaggttcaccgcgtcctggtccgcgcgcgggtcgcccacgcgcacgatgcggctacccttcgcatcccacacgaattcgccgtcttcgaacaccagctggatcgtgccatcgaccagctgctggatctgcatttccagcgcgtcgaagcccttttcgatggtttcggcgtggaaggcgccctggttggtgatgtcggtttcctgggtgtacggcatcgtgcgcagcagcagcagcatttcgtcggcggccggcggcgtgtgcatcgtgacgcgggtgcccgactcgtaccccagcttttccacgtcgaaactggcgctgggcaccagggtcatcgtgttgcccttcaccaggaaggcgtacacgtgcgcgcgcgcataggccatcggcccgttgaacacctgggtgacgccgttgccctggtattcgcggcggcggctgttggcggaaacggtcattatttgggttccttcttggggccggtcaggtattcgtatggcgacacgtcgcggccgtccgcgcgcgccgcgatggcgtcgatggtcttattgacctgggtggacggcaagcccagcgtgacgcccgccgcggacactgccgccttcgccacgcccttgtccaggttcacttcgccgtcctcgccgggggtcagcttttccagcagttcggcgtaggcgcgccaggcgccggccaccacgccgctggaatcgtagccgcggaactggtcaaccagcacgccgccgccggggatcacgccgaagaacgtggacagcgcatccttgatcgcccattcgcccaggtcatcccacaggccgtcgtcgtcgtcatcgttcggcagcttcgcggtcagggccgcggtcagcaggccttccacggagaacagcatcaccatgtcggcggcccacttcatcgcctggcgcgggtttcgcagattcgccttgcgggtctgttcgtaggccagattcccctttgcgatcatgtagccttgcagggcggtggtggccttgatccattccgtttggcgcacgttgtcgcccagcgtgccgcgctgcagcggcgacttgtcgatgaactcgcccgaaccctgggcgcgcgtcaccacgtcgtcggcataggcgcgggcgcggcccacgtcgttgccgaacttggccatgcccgcctgttcggcggccagccaggtcacggtatccaccagcccctgcacgcggccgatcatccagtaaccgaaccggatgctggcggccttccccgcggcgaacctgccggcttccgcatccatcacggtctgcaccgcttcgatgtgcgtgcgcaggcggctgtccatgtacggcgacgcctcgcgcacgtagcgcgtcatcgcgcgcggcttgcccaggtactggccgatgccagccatggtgtggccctggccgatggtgacgatggtgggcacaacgcccgacagctgcagcagcgcgctggtgactttgaaggtcagcaccgacgcggtgaagttctggcgggcggcgcgcatggcgcgttcgtgccacacgcgcggcccaatctcgccggccgccgcgtccttcaaccacacttccagcgcctggcggtactcctgggtgccggtgctgtccacggcttccttgaactcctggccgttcagcacgttgtggacgtagttgaccgcatcgcccaggtggacatcgcgcagcacgtcgcgcaggtgctgctgcaccacgcccgtgtccaggcgcacggtgcgcccgcccgacccgacacgttcgatggtgtggccgttgcgggtcgcagccttcgcggtgcggccggtgcggatgctgttatagaagtcgtccgcttcgtccttcatggtcttgacggaatcggattcgtacttcaacgggtaatagccgccagggatctgcagcgttttcccgtcgctggtctgcacggtgaaggcgctggcctgcacgcgctccggcaccaggccggtgcgacgcttctgcgcgtcggcaatggccggccactgcgaatcgatcaagcgccacacgtcttccacgaacgcccagtcgcgcgaatccagcttcgacagcagggcgttcacctgttccggcgacatgcgcccgcgcgcctgggtcaggatcgcttcgcggttgccggcattgccccagttcagcgccaggccaagcaggcgggacttgctccacaggtcgccgttcacttcgggcatcggcacgcgctcggagaagccgcggatttccgccttgctgtagtgcttcacgtagacctgggccagttcgtcctgcgcctgctgcagcgccgggttcagccggttgttcaccgcgtcgcgcatcacgcccacggtgttcatccagatggcgccctgatccttgaacccatccagttcgcgggccatgtcggtggccgtggcctggatcacgcggccctgcatgaaggcctggcgcagccggtccttcggcccgcggtcgcccgtggtgatcgggcgcgcttcgtgcgcagcggccaggctggcggccatggcggcatccacttccgcggcatcgcgcacttcgccggccagcagcagcttgcccttcaatcgcgccaggtgatcgatggaacggatggcatcgcgcagcgtggccaggtccgccacggtcatttcgcggtacggaatggtgaacgcttcgtccatgatcttgggcggcaggttcacgtcgatccccttctgcgcctgcacttcgatccaggtggccagcgaggaacggcggtcggccgccttgtcgctgatcttgcggaagtcgaagcggtccagcaggccatccacctggtcgaggtagtcggcgccagccttgcccaggcgtgcgcgggtcttcgtctcgccgaacttggccaggtacttcgcggtgcgtgcggcctcatcgcgcgcgcgcacggcttcgcggaacagttcgaagttcagcagctgccggcggcgcgcggccagggcgttgccccagtcctgcttcgccgcggcttcgaaggcctcacgcccggcccttgcttcggccgaacggtaggtggccggctgcaggtggcgcagcttcttgtcctggatgatctggcgagccacgcccttgatgaccgcggcctgcgatacctggcggccgttgacgtgctgttccagcgcgcgaatctcgcgcaccatcacgtcggcctggcggtcccggtgcgccgcgatcatggcgcggtcgggcagcgtgccatccgtcatcggatccgggtggcggtccttcatgcgcgcttccgtctcgctggccacagcgtcggccaggcgcggcgcgttcaccagcgattcgatcaattcgcggccggacccgaacccgtagatggccgcggcttcgtcgccgcgcacgccgccttccaccgaatacatgccgaccaggttgcgcaggaaggactggccgaacttgtccagcagttcgtccttcgacagcttgacccgcagttcgtccggggccaggtcgccgttcggcagcttcccgttgcgcagcaggcgctgggcgcgatacaccggcagattgcggacctcttccagcacctgggcgcgcacttcgcgcttctcgcggttgtaccaggcctgttgctcgcggcgctcggccagcagcacttcggccgccacggtggcttcggcgtcggcgcgcgcggtgttcaccgcttcgttgtaggcctgcagctgttcgaaggtcatgcccacagccatgccatcggcaatcagcgcgccctggtactggccggcgcgggcgtcttcaatctcggcatcgctggccacgatgcggtccatgacgttgcgcacgtcatcggtcagttccacgttgaggctgcgcacgctgcggtacagcgcggtcagccacaccttgaacgcggcgaacgtgcggcgcagcgcagacgacggcgccttgccctcgcgcaggtaggcttcgaagccgcgggcgaactgttcgtgctggtcaacggtgaacgcggcgccggcctcgcggcccagccaggtgttcagggtggccatgtcgttggtgatctgcgcgggcgcgccatcacgcgcggccaggtcattcagcacttccaggtacacgtgccccatttcgtgcatgaaggtgctggcgtccatgcctttcagcagttcgatgttgaacacccgcgcgccgggcacaccttcgaacgtgacggcgccgcgcggcttctcgccgccctggttcagcgccgcggcgtcggtgatcggaacgcccagccggttggcctcgctcatctgcgcgaagttggccgcgcgcgggttggcctgggcgaagtccaccaggtcgctggtcgattcgatcaaggcatccagcgcggtgcgttcctgcccggtcacgcccagcatcgtcgcaatggcgtccttgaaccactgccaggccgtgcgcgattcctcgcggccagccggcgccggcacggtggcaagccattcctggaaccgcttgtcggtcatgccgtaggtcagcagttccttgatgttcgacagtgggccgcgcggatcctgcagcgtggcgcgcagcgccgccggcacatcggcgccatcggtttccatgcctgcgaagtgggcctgggcagcgcccagcaagtcgttgaactcggccacggcgcgcgccacggtcgtgttcgaccggcgcagggtcgggctggtcatcatcgccgacgtgacgccatgcaggacttcgtgcagcaccacggacgggaccgcctggtggatccagatttcgttcgtggtgttgttgtagatgccggcggcgttggcgttggccggtgccgccaccatcgtcacgttcaggtcgggcgtgatttcagccaggcgcagcgcaagcgcggcctggtcggcatcgatcccttcctgggtggcgatgccctgcagcatcttggccaggtcgccatcggccaccgcctgatccaccagcgcgcgcgtcgcggcgctttccggccggccgctcggcccggccaccaggtcgcgcacggcgtagtccacaccatcggattcgaccggctggccctgttccagggtccggttcgcgtaccccagcgcctggcgtgccgtcgcgttgtcggtctgctgcaggtcgatgccgcgctggtcaagctcatcctgcaggcccagggcgctgtcacggaacgcggcgcgctcggcgttcatcgctgccggccggtacaccgggttcccgccaagatcctgggcgagcatgtccagcagcgtgttgatgtccggcgcgtcggcgtcgtaggcgccttcctgctggttcgtcggtgcctgggtgatgaagccttcctggtaggcccacaccagcgcatcgtccaggctcatacctgccaggttgttgaccaggccggggtgcgccttcgccgcgtccatgttggccagttcgccgccggagtcgcgcaggccgccggccgcg

SEQ ID NO: 2 - DNA, 20 bp, synthetic construct
  source 1..20: mol_type = other DNA
gcgcagtcatgagatcgaga

SEQ ID NO: 3 - DNA, 20 bp, synthetic construct
  source 1..20: mol_type = other DNA
gttgagtgcaccgagagtga

SEQ ID NO: 4 - DNA, 20 bp, synthetic construct
  source 1..20: mol_type = other DNA
tgggtcacttcggtgttacg

SEQ ID NO: 5 - DNA, 20 bp, synthetic construct
  source 1..20: mol_type = other DNA
gtggtgaaaggtgcggtttc

SEQ ID NO: 6 - DNA, 20 bp, synthetic construct
  source 1..20: mol_type = other DNA
cgtagtcgcgattgtcggta

SEQ ID NO: 7 - DNA, 20 bp, synthetic construct
  source 1..20: mol_type = other DNA
accactgctgacgttcgatt

SEQ ID NO: 8 - DNA, 20 bp, synthetic construct
  source 1..20: mol_type = other DNA
gctaccggtacgactacgtg

SEQ ID NO: 9 - DNA, 20 bp, synthetic construct
  source 1..20: mol_type = other DNA
gatctggaaacagccgtcca

SEQ ID NO: 10 - DNA, 19 bp, synthetic construct
  source 1..19: mol_type = other DNA
tttcggtggcttggatttt

SEQ ID NO: 11 - DNA, 20 bp, synthetic construct
  source 1..20: mol_type = other DNA
atttgcgagaagtacaactg

SEQ ID NO: 12 - DNA, 20 bp, synthetic construct
  source 1..20: mol_type = other DNA
atcccctttgcatcttcaat

SEQ ID NO: 13 - DNA, 20 bp, synthetic construct
  source 1..20: mol_type = other DNA
ttccgtcatctaagggaatc

SEQ ID NO: 14 - DNA, 20 bp, synthetic construct
  source 1..20: mol_type = other DNA
taagcccttcgtaaagttct

SEQ ID NO: 15 - DNA, 20 bp, synthetic construct
  source 1..20: mol_type = other DNA
aagcattgaaaaacgaaacg

SEQ ID NO: 16 - DNA, 21 bp, synthetic construct
  source 1..21: mol_type = other DNA
actaggagaagattagatggc

SEQ ID NO: 17 - DNA, 16 bp, synthetic construct
  source 1..16: mol_type = other DNA
ctggtccgtaagggtg

SEQ ID NO: 18 - DNA, 20 bp, synthetic construct
  source 1..20: mol_type = other DNA
gatatacgagcaacgtcttc

SEQ ID NO: 19 - DNA, 20 bp, synthetic construct
  source 1..20: mol_type = other DNA
atttgcgagaagtacaactg

SEQ ID NO: 20 - DNA, 20 bp, synthetic construct
  source 1..20: mol_type = other DNA
gttattgcgacggttaaaga

SEQ ID NO: 21 - DNA, 20 bp, synthetic construct
  source 1..20: mol_type = other DNA
tggattaaatactacgccga

SEQ ID NO: 22 - DNA, 20 bp, synthetic construct
  source 1..20: mol_type = other DNA
ctggcaaaacaacctcatta

SEQ ID NO: 23 - DNA, 20 bp, synthetic construct
  source 1..20: mol_type = other DNA
agttaccacgaggatttcat

SEQ ID NO: 24 - DNA, 19 bp, synthetic construct
  source 1..19: mol_type = other DNA
gtagatgttcggttcggta

SEQ ID NO: 25 - DNA, 20 bp, synthetic construct
  source 1..20: mol_type = other DNA
caagccaattcacatcgtag

SEQ ID NO: 26 - DNA, 20 bp, synthetic construct
  source 1..20: mol_type = other DNA
attctgtttcaacaaccctg

SEQ ID NO: 27 - DNA, 20 bp, synthetic construct
  source 1..20: mol_type = other DNA
cagacatccaggaacttttc

SEQ ID NO: 28 - DNA, 20 bp, synthetic construct
  source 1..20: mol_type = other DNA
catacctacgatatacggca

SEQ ID NO: 29 - DNA, 20 bp, synthetic construct
  source 1..20: mol_type = other DNA
gactactcgctctacatcaa

SEQ ID NO: 30 - DNA, 20 bp, synthetic construct
  source 1..20: mol_type = other DNA
atggcctttcttcattcttg

SEQ ID NO: 31 - DNA, 20 bp, synthetic construct
  source 1..20: mol_type = other DNA
agaaaatatccgggtgtgat

SEQ ID NO: 32 - DNA, 20 bp, synthetic construct
  source 1..20: mol_type = other DNA
tagattgtgattcacgcaac

SEQ ID NO: 33 - DNA, 20 bp, synthetic construct
  source 1..20: mol_type = other DNA
gaagacgaaaaggcaaaaac

SEQ ID NO: 34 - DNA, 20 bp, synthetic construct
  source 1..20: mol_type = other DNA
atattgaactccgaagtcgt

SEQ ID NO: 35 - DNA, 19 bp, synthetic construct
  source 1..19: mol_type = other DNA
ctaccaaactgggggatag